European Patent Application EP 4 173 637 A1, published May 3, 2023. Title: FORMULATION FOR ANTI-FcRn ANTIBODY. Applicant: Hanall Biopharma Co., Ltd. The sequence listing filed with the application follows.

SEQUENCE LISTING (10 sequences)

SEQ ID NO: 1 - protein, 450 aa, Artificial Sequence
  HL161_Heavy chain
QLLLQESGPGLVKPSETLSLTCTVSGGSLSSSFSYWVWIRQPPGKGLEWIGTIYYSGNTYYNPSLKSRLTISVDTSKNHFSLKLSSVTAADTAVYYCARRAGILTGYLDSWGQGTLVTVSSASTKGPSVFPLAPSSKSTSGGTAALGCLVKDYFPEPVTVSWNSGALTSGVHTFPAVLQSSGLYSLSSVVTVPSSSLGTQTYICNVNHKPSNTKVDKRVEPKSCDKTHTCPPCPAPEAAGGPSVFLFPPKPKDTLMISRTPEVTCVVVDVSHEDPEVKFNWYVDGVEVHNAKTKPREEQYNSTYRVVSVLTVLHQDWLNGKEYKCKVSNKALPAPIEKTISKAKGQPREPQVYTLPPSREEMTKNQVSLTCLVKGFYPSDIAVEWESNGQPENNYKTTPPVLDSDGSFFLYSKLTVDKSRWQQGNVFSCSVMHEALHNHYTQKSLSLSPG

SEQ ID NO: 2 - protein, 214 aa, Artificial Sequence
  HL161_Light chain
SYVLTQSPSVSVAPGQTARITCGGNNIGSKSVHWYQQKPGQAPVLVVYDDSDRPSGIPERFSASNSGNTATLTISRVEAGDEADYYCQVWDSSSDHVVFGGGTKLTVLGQPKAAPSVTLFPPSSEELQANKATLVCLISDFYPGAVTVAWKADSSPVKAGVETTTPSKQSNNKYAASSYLSLTPEQWKSHRSYSCQVTHEGSTVEKTVAPTECS

SEQ ID NO: 3 - DNA, 1350 bp, Artificial Sequence
  polynucleotides coding HL161 heavy chain
cagctgctgctgcaagaatccggccctggcctggtgaaaccctccgagacactgtccctgacctgcaccgtgtccggcggctccctgtcctccagcttctcctactgggtctggatccggcagccccctggcaagggcctggaatggatcggcaccatctactactccggcaacacctactacaaccccagcctgaagtcccggctgaccatctccgtggacacctccaagaaccacttcagcctgaagctgtcctccgtgaccgccgctgacaccgccgtgtactactgtgccagaagggccggcatcctgaccggctacctggactcttggggccagggcaccctggtgacagtgtcctccgcctccaccaagggcccctccgtgttccctctggccccctccagcaagtccacctctggcggcaccgctgccctgggctgtctggtgaaagactacttccccgagcccgtgaccgtgtcctggaactctggcgccctgacctccggcgtgcacaccttccctgccgtgctgcagtcctccggcctgtactccctgtccagcgtggtgaccgtgccctccagctctctgggcacccagacctacatctgcaacgtgaaccacaagccctccaacaccaaggtggacaagcgggtggaacccaagtcctgcgacaagacccacacctgtcccccctgtcctgcccctgaagctgctggcggccctagcgtgttcctgttccccccaaagcccaaggacaccctgatgatctcccggacccccgaagtgacctgcgtggtggtggacgtgtcccacgaggaccctgaagtgaagttcaattggtacgtggacggcgtggaagtgcacaacgccaagaccaagcccagagaggaacagtacaactccacctaccgggtggtgtccgtgctgaccgtgctgcaccaggactggctgaacggcaaagagtacaagtgcaaggtctccaacaaggccctgcctgcccccatcgaaaagaccatctccaaggccaagggccagccccgcgagccccaggtgtacacactgccccctagccgggaagagatgaccaagaaccaggtgtccctgacatgcctggtgaagggcttctacccctccgacattgccgtggaatgggagtccaacggccagcccgagaacaactacaagaccaccccccctgtgctggactccgacggctcattcttcctgtactccaagctgaccgtggacaagtcccggtggcagcagggcaacgtgttctcctgctccgtgatgcacgaggccctgcacaaccactacacccagaagtccctgtccctgagccccggc

SEQ ID NO: 4 - DNA, 642 bp, Artificial Sequence
  polynucleotides coding HL161 light chain
tcttacgtgctgacccagtccccctccgtgtccgtggctcctggccagaccgccagaatcacctgtggcggcaacaacatcggctccaagtccgtgcactggtatcagcagaagcccggccaggcccccgtgctggtggtgtacgacgactccgaccggccctctggcatccctgagcggttctccgcctccaactccggcaacaccgccaccctgaccatctccagagtggaagccggcgacgaggccgactactactgccaagtgtgggactcctcctccgaccacgtggtgttcggcggaggcaccaagctgaccgtgctgggccagcctaaggccgctccctccgtgaccctgttccccccatcctccgaggaactgcaggccaacaaggccaccctggtctgcctgatctccgacttctaccctggcgccgtgaccgtggcctggaaggccgacagctctcctgtgaaggccggcgtggaaaccaccaccccctccaagcagtccaacaacaaatacgccgcctcctcctacctgtccctgacccccgagcagtggaagtcccaccggtcctacagctgccaagtgacacacgagggctccaccgtggaaaagaccgtggcccctaccgagtgctcc

SEQ ID NO: 5 - protein, 5 aa, Artificial Sequence
  HL161_Hv CDR1
FSYWV

SEQ ID NO: 6 - protein, 16 aa, Artificial Sequence
  HL161_Hv CDR2
TIYYSGNTYYNPSLKS

SEQ ID NO: 7 - protein, 11 aa, Artificial Sequence
  HL161_Hv CDR3
RAGILTGYLDS

SEQ ID NO: 8 - protein, 11 aa, Artificial Sequence
  HL161_Lv CDR1
GGNNIGSKSVH

SEQ ID NO: 9 - protein, 7 aa, Artificial Sequence
  HL161_Lv CDR2
DDSDRPS

SEQ ID NO: 10 - protein, 11 aa, Artificial Sequence
  HL161_Lv CDR3
QVWDSSSDHVV